European Patent Specification EP 3 555 281 B1, published October 22, 2025. Title: NOVEL PROTEASES AND USES THEREOF. Applicant: CARBIOS. The sequence listing filed with the application follows.

SEQUENCE LISTING (44 sequences)

SEQ ID NO: 1 - protein, 278 aa, Thermus sp. strain Rt41A [sequence omitted]

SEQ ID NO: 2 - DNA, 1170 bp, artificial sequence
  sequence encoding propeptide and protease
aaccctcccgctgcttccacccaggaagctcccctgctgggcctggaggctcctgaggctatccccggccgatacattgtcgtctacaaggagaacgctgacgtgctgcctgctctggaggctctcaaggctgctctggagcctggtctcatgcagcctcagggactgcaggctcaggctctccgaaccctcggcctggagggtgctcgagtggacaaggtctacaccgctgctctgcgaggtgtggctgtggaggtgcctgaccaggagctggctcgactccgacaggacccccgagtggcttacatcgaggccgaccaggaagtccgagctttcgccgtgcagtctcctgctacctggggtctggaccgaattgaccagcgaaccctccccctggacggacgatacacctacaccgctaccggtgctggagtccacgcctacgtcgtggacaccggcatcctgctctcccaccaggagttcaccggtcgaatcggcaagggttacgacgctattacccccggcggttctgctcaggactgcaacggacacggcacccacgtggctggcaccattggaggcaccacctacggagtggctaagggtgtgaccctgcaccccgtccgagtgctcgactgtaacggttccggatctaactcctctgtcatcgctggtctggactgggtgacccagaaccacgtcaagcccgccgtgattaacatgtccctgggtggaggcgcttctaccgctctggacaccgccgtcatgaacgctatcaacgctggtgtgaccgtggtggtggctgctggtaacgacaaccgagacgcttgtttctactctcccgctcgagtcaccgctgctattaccgtgggagctaccacctctaccgactaccgagcctccttctctaactacggtcgatgtctcgacctgttcgcccccggacagtccatcacctctgcttggtacacctcctctaccgccaccaacaccatttccggaacctctatggctacccctcacgtgaccggtgccgctgccctctacctgcagtggtaccctaccgctaccccttcccaggtggcttctgccctgctctactacgctacccccaacgtggtcaagaacgccggccgatactcccccaacctgctcctctacacccccttc

SEQ ID NO: 3 - DNA, 23 bp, artificial sequence
  N102S forward primer
ctcgactgtagcggttccggatc

SEQ ID NO: 4 - DNA, 23 bp, artificial sequence
  N102S reverse primer
gatccggaaccgctacagtcgag

SEQ ID NO: 5 - DNA, 24 bp, artificial sequence
  S106T forward primer
tccggaactaactcctctgtcatc

SEQ ID NO: 6 - DNA, 24 bp, artificial sequence
  S106T reverse primer
ggagttagttccggaaccgttaca

SEQ ID NO: 7 - DNA, 20 bp, artificial sequence
  N107T forward primer
ccggatctacctcctctgtc

SEQ ID NO: 8 - DNA, 20 bp, artificial sequence
  N107T reverse primer
gacagaggaggtagatccgg

SEQ ID NO: 9 - DNA, 22 bp, artificial sequence
  D160E forward primer
gctggtaacgaaaaccgagacg

SEQ ID NO: 10 - DNA, 22 bp, artificial sequence
  D160E reverse primer
cgtctcggttttcgttaccagc

SEQ ID NO: 11 - DNA, 35 bp, artificial sequence
  Y167R forward primer
cgagacgcttgtttccgctctcccgctcgagtcac

SEQ ID NO: 12 - DNA, 33 bp, artificial sequence
  Y167R reverse primer
gaaacaagcgtctcggttgtcgttaccagcagc

SEQ ID NO: 13 - DNA, 38 bp, artificial sequence
  D160E+Y167R forward primer
taacgaaaaccgagacgcttgtttccgctctcccgctc

SEQ ID NO: 14 - DNA, 40 bp, artificial sequence
  D160E+Y167R reverse primer
gggagagcggaaacaagcgtctcggttttcgttaccagca

SEQ ID NO: 15 - DNA, 33 bp, artificial sequence
  N102S+S106T+N107T forward primer
tgtagcggttccggaactacctcctctgtcatc

SEQ ID NO: 16 - DNA, 35 bp, artificial sequence
  N102S+S106T+N107T reverse primer
aggaggtagttccggaaccgctacagtcgagcact

SEQ ID NO: 17 - DNA, 24 bp, artificial sequence
  N102F forward
gactgtttcggttccggatctaac

SEQ ID NO: 18 - DNA, 24 bp, artificial sequence
  N102F forward mutated
gactgtttcggttccggaactacc

SEQ ID NO: 19 - DNA, 23 bp, artificial sequence
  N102F reverse
ggaaccgaaacagtcgagcactc

SEQ ID NO: 20 - DNA, 24 bp, artificial sequence
  S104L forward
aacggtctcggatctaactcctct

SEQ ID NO: 21 - DNA, 24 bp, artificial sequence
  S104L reverse
agatccgagaccgttacagtcgag

SEQ ID NO: 22 - DNA, 24 bp, artificial sequence
  N107I forward
ggatctatctcctctgtcatcgct

SEQ ID NO: 23 - DNA, 24 bp, artificial sequence
  N107I reverse
agaggagatagatccggaaccgtt

SEQ ID NO: 24 - DNA, 29 bp, artificial sequence
  S104L+N107I forward
aacggtctcggatctatctcctctgtcat

SEQ ID NO: 25 - DNA, 29 bp, artificial sequence
  S104L+N107I reverse
agaggagatagatccgagaccgttacagt

SEQ ID NO: 26 - DNA, 30 bp, artificial sequence
  N102F+S104L forward
gactgtttcggtctcggatctaactcctct

SEQ ID NO: 27 - DNA, 30 bp, artificial sequence
  N102F+S104L reverse
agatccgagaccgaaacagtcgagcactcg

SEQ ID NO: 28 - DNA, 30 bp, artificial sequence
  N102F+S104L+N107I forward
tgtttcggtctcggatctatctcctctgtc

SEQ ID NO: 29 - DNA, 30 bp, artificial sequence
  N102F+S104L+N107I reverse
aggagatagatccgagaccgaaacagtcga

SEQ ID NO: 30 - DNA, 30 bp, artificial sequence
  N102F+S104L+S106T+N107I forward
tgtttcggtctcggaactatctcctctgtc

SEQ ID NO: 31 - DNA, 30 bp, artificial sequence
  N102F+S104L+S106T+N107I reverse
aggagatagttccgagaccgaaacagtcga

SEQ ID NO: 32 - DNA, 24 bp, artificial sequence
  G132I forward
tccctgattggaggcgcttctacc

SEQ ID NO: 33 - DNA, 24 bp, artificial sequence
  G132I reverse
agcgcctccaatcagggacatgtt

SEQ ID NO: 34 - DNA, 24 bp, artificial sequence
  G134K forward
ggtggaaaggcttctaccgctctg

SEQ ID NO: 35 - DNA, 24 bp, artificial sequence
  G134K reverse
ggtagaagcctttccacccaggga

SEQ ID NO: 36 - DNA, 33 bp, artificial sequence
  N102S+S106T forward
tgtagcggttccggaactaactcctctgtcatc

SEQ ID NO: 37 - DNA, 35 bp, artificial sequence
  N102S+S106T reverse
aggagttagttccggaaccgctacagtcgagcact

SEQ ID NO: 38 - DNA, 33 bp, artificial sequence
  N102S+N107T forward
tgtagcggttccggatctacctcctctgtcatc

SEQ ID NO: 39 - DNA, 35 bp, artificial sequence
  N102S+N107T reverse
aggaggtagatccggaaccgctacagtcgagcact

SEQ ID NO: 40 - DNA, 33 bp, artificial sequence
  S106T+N107T forward
tgtaacggttccggaactacctcctctgtcatc

SEQ ID NO: 41 - DNA, 35 bp, artificial sequence
  S106T+N107T reverse
aggaggtagttccggaaccgttacagtcgagcact

SEQ ID NO: 42 - protein, 112 aa, artificial sequence
  propeptide
NPPAASTQEAPLLGLEAPEAIPGRYIVVYKENADVLPALEALKAALEPGLMQPQGLQAQALRTLGLEGARVDKVYTAALRGVAVEVPDQELARLRQDPRVAYIEADQEVRAF

SEQ ID NO: 43 - protein, 22 aa, artificial sequence
  PelB signal peptide
MKYLLPTAAAGLLLLAAQPAMA

SEQ ID NO: 44 - protein, 8 aa, artificial sequence
  6xhistidine tag
LEHHHHHH